European Patent Application EP 4 524 243 A1, published March 19, 2025. Title: Reprogrammed functional fragment of recombinant oncolytic virus, combination, and application thereof. Applicant: NEUREGEN BIOTHERAPEUTICS (SHANGHAI) CO. LTD. Application CN PCT/CN2023/093135, filed May 10, 2023. The sequence listing filed with the application follows.

SEQUENCE LISTING (19 sequences)

SEQ ID NO: 1 - protein, 356 aa, Homo sapiens
MTKSYSESGLMGEPQPQGPPSWTDECLSSQDEEHEADKKEDDLETMNAEEDSLRNGGEEEDEDEDLEEEEEEEEEDDDQKPKRRGPKKKKMTKARLERFKLRRMKANARERNRMHGLNAALDNLRKVVPCYSKTQKLSKIETLRLAKNYIWALSEILRSGKSPDLVSFVQTLCKGLSQPTTNLVAGCLQLNPRTFLPEQNQDMPPHLPTASASFPVHPYSYQSPGLPSPPYGTMDSSHVFHVKPPPHAYSAALEPFFESPLTDCTSPSFDGPLSPPLSINGNFSFKHEPSAEFEKNYAFTMHYPAATLAGAQSHGSIFSGTAAPRCEIPIDNIMSFDSHSHHERVMSAQLNAIFHD

SEQ ID NO: 2 - protein, 357 aa, Mus musculus
MTKSYSESGLMGEPQPQGPPSWTDECLSSQDEEHEADKKEDELEAMNAEEDSLRNGGEEEEEDEDLEEEEEEEEEEEDQKPKRRGPKKKKMTKARLERFKLRRMKANARERNRMHGLNAALDNLRKVVPCYSKTQKLSKIETLRLAKNYIWALSEILRSGKSPDLVSFVQTLCKGLSQPTTNLVAGCLQLNPRTFLPEQNPDMPPHLPTASASFPVHPYSYQSPGLPSPPYGTMDSSHVFHVKPPPHAYSAALEPFFESPLTDCTSPSFDGPLSPPLSINGNFSFKHEPSAEFEKNYAFTMHYPAATLAGPQSHGSIFSSGAAAPRCEIPIDNIMSFDSHSHHERVMSAQLNAIFHD

SEQ ID NO: 3 - DNA, 1071 bp, Homo sapiens
  source 1..1071: mol_type = genomic DNA
atgaccaaatcgtacagcgagagtgggctgatgggcgagcctcagccccaaggtcctccaagctggacagacgagtgtctcagttctcaggacgaggagcacgaggcagacaagaaggaggacgacctcgaaaccatgaacgcagaggaggactcactgaggaacgggggagaggaggaggacgaagatgaggacctggaagaggaggaagaagaggaagaggaggatgacgatcaaaagcccaagagacgcggccccaaaaagaagaagatgactaaggctcgcctggagcgttttaaattgagacgcatgaaggctaacgcccgggagcggaaccgcatgcacggactgaacgcggcgctagacaacctgcgcaaggtggtgccttgctattctaagacgcagaagctgtccaaaatcgagactctgcgcttggccaagaactacatctgggctctgtcggagatcctgcgctcaggcaaaagcccagacctggtctccttcgttcagacgctttgcaagggcttatcccaacccaccaccaacctggttgcgggctgcctgcaactcaatcctcggacttttctgcctgagcagaaccaggacatgcccccccacctgccgacggccagcgcttccttccctgtacacccctactcctaccagtcgcctgggctgcccagtccgccttacggtaccatggacagctcccatgtcttccacgttaagcctccgccgcacgcctacagcgcagcgctggagcccttctttgaaagccctctgactgattgcaccagcccttcctttgatggacccctcagcccgccgctcagcatcaatggcaacttctctttcaaacacgaaccgtccgccgagtttgagaaaaattatgcctttaccatgcactatcctgcagcgacactggcaggggcccaaagccacggatcaatcttctcaggcaccgctgcccctcgctgcgagatccccatagacaatattatgtccttcgatagccattcacatcatgagcgagtcatgagtgcccagctcaatgccatatttcatgattag

SEQ ID NO: 4 - DNA, 1074 bp, Mus musculus
  source 1..1074: mol_type = genomic DNA
atgaccaaatcatacagcgagagcgggctgatgggcgagcctcagccccaaggtcccccaagctggacagatgagtgtctcagttctcaggacgaggaacacgaggcagacaagaaagaggacgagcttgaagccatgaatgcagaggaggactctctgagaaacgggggagaggaggaggaggaagatgaggatctagaggaagaggaggaagaagaagaggaggaggaggatcaaaagcccaagagacggggtcccaaaaagaaaaagatgaccaaggcgcgcctagaacgttttaaattaaggcgcatgaaggccaacgcccgcgagcggaaccgcatgcacgggctgaacgcggcgctggacaacctgcgcaaggtggtaccttgctactccaagacccagaaactgtctaaaatagagacactgcgcttggccaagaactacatctgggctctgtcagagatcctgcgctcaggcaaaagccctgatctggtctccttcgtacagacgctctgcaaaggtttgtcccagcccactaccaatttggtcgccggctgcctgcagctcaaccctcggactttcttgcctgagcagaacccggacatgcccccgcatctgccaaccgccagcgcttccttcccggtgcatccctactcctaccagtcccctggactgcccagcccgccctacggcaccatggacagctcccacgtcttccacgtcaagccgccgccacacgcctacagcgcagctctggagcccttctttgaaagccccctaactgactgcaccagcccttcctttgacggacccctcagcccgccgctcagcatcaatggcaacttctctttcaaacacgaaccatccgccgagtttgaaaaaaattatgcctttaccatgcactaccctgcagcgacgctggcagggccccaaagccacggatcaatcttctcttccggtgccgctgcccctcgctgcgagatccccatagacaacattatgtctttcgatagccattcgcatcatgagcgagtcatgagtgcccagcttaatgccatctttcacgattag

SEQ ID NO: 5 - protein, 443 aa, Homo sapiens
MATAASNHYSLLTSSASIVHAEPPGGMQQGAGGYREAQSLVQGDYGALQSNGHPLSHAHQWITALSHGGGGGGGGGGGGGGGGGGGGGDGSPWSTSPLGQPDIKPSVVVQQGGRGDELHGPGALQQQHQQQQQQQQQQQQQQQQQQQQQRPPHLVHHAANHHPGPGAWRSAAAAAHLPPSMGASNGGLLYSQPSFTVNGMLGAGGQPAGLHHHGLRDAHDEPHHADHHPHPHSHPHQQPPPPPPPQGPPGHPGAHHDPHSDEDTPTSDDLEQFAKQFKQRRIKLGFTQADVGLALGTLYGNVFSQTTICRFEALQLSFKNMCKLKPLLNKWLEEADSSSGSPTSIDKIAAQGRKRKKRTSIEVSVKGALESHFLKCPKPSAQEITSLADSLQLEKEVVRVWFCNRRQKEKRMTPPGGTLPGAEDVYGGSRDTPPHHGVQTPVQ

SEQ ID NO: 6 - protein, 445 aa, Mus musculus
MATAASNHYSLLTSSASIVHAEPPGGMQQGAGGYREAQSLVQGDYGALQSNGHPLSHAHQWITALSHGGGGGGGGGGGGGGGGGGGGGDGSPWSTSPLGQPDIKPSVVVQQGGRGDELHGPGALQQQHQQQQQQQQQQQQQQQQQQQQQQQRPPHLVHHAANHHPGPGAWRSAAAAAHLPPSMGASNGGLLYSQPSFTVNGMLGAGGQPAGLHHHGLRDAHDEPHHADHHPHPHSHPHQQPPPPPPPQGPPGHPGAHHDPHSDEDTPTSDDLEQFAKQFKQRRIKLGFTQADVGLALGTLYGNVFSQTTICRFEALQLSFKNMCKLKPLLNKWLEEADSSSGSPTSIDKIAAQGRKRKKRTSIEVSVKGALESHFLKCPKPSAQEITSLADSLQLEKEVVRVWFCNRRQKEKRMTPPGGTLPGAEDVYGGSRDTPPHHGVQTPVQ

SEQ ID NO: 7 - DNA, 1332 bp, Homo sapiens
  source 1..1332: mol_type = genomic DNA
atggcgaccgcagcgtctaaccactacagcctgctcacctccagcgcctccatcgtgcacgccgagccgcccggcggcatgcagcagggcgcggggggctaccgcgaagcgcagagcctggtgcagggcgactacggcgctctgcagagcaacggacacccgctcagccacgctcaccagtggatcaccgcgctgtcccacggcggcggcggcgggggcggtggcggcggcggggggggcgggggcggcggcgggggcggcggcgacggctccccgtggtccaccagccccctgggccagccggacatcaagccctcggtggtggtgcagcagggcggccgcggagacgagctgcacgggccaggcgccctgcagcagcagcatcagcagcagcaacagcaacagcagcagcaacagcagcaacagcagcagcagcagcagcaacagcggccgccgcatctggtgcaccacgccgctaaccaccacccgggacccggggcatggcggagcgcggcggctgcagcgcacctcccaccctccatgggagcgtccaacggcggcttgctctactcgcagcccagcttcacggtgaacggcatgctgggcgccggcgggcagccggccggtctgcaccaccacggcctgcgggacgcgcacgacgagccacaccatgccgaccaccacccgcacccgcactcgcacccacaccagcagccgccgcccccgccgcccccgcagggtccgcctggccacccaggcgcgcaccacgacccgcactcggacgaggacacgccgacctcggacgacctggagcagttcgccaagcagttcaagcagcggcggatcaaactgggatttacccaagcggacgtggggctggctctgggcaccctgtatggcaacgtgttctcgcagaccaccatctgcaggtttgaggccctgcagctgagcttcaagaacatgtgcaagctgaagcctttgttgaacaagtggttggaggaggcggactcgtcctcgggcagccccacgagcatagacaagatcgcagcgcaagggcgcaagcggaaaaagcggacctccatcgaggtgagcgtcaagggggctctggagagccatttcctcaaatgccccaagccctcggcccaggagatcacctccctcgcggacagcttacagctggagaaggaggtggtgagagtttggttttgtaacaggagacagaaagagaaaaggatgacccctcccggagggactctgccgggcgccgaggatgtgtacggggggagtagggacactccaccacaccacggggtgcagacgcccgtccagtga

SEQ ID NO: 8 - DNA, 1338 bp, Mus musculus
  source 1..1338: mol_type = genomic DNA
atggcgaccgcagcgtctaaccactacagcctgctcacctccagcgcctccatcgtacatgccgagccgcctggcggcatgcagcagggcgcagggggctaccgcgaggcgcagagcctggtgcagggcgactacggcgcgctgcagagcaacgggcacccgctcagccacgctcaccagtggatcaccgcgctgtcccacggcggcggcggcgggggcggcggcggcggtggaggaggcgggggaggcggcgggggaggcggcgacggctccccgtggtccaccagccccctaggccagccggacatcaagccctcggtggtggtacagcagggtggccgaggcgacgagctgcacgggccaggagcgctgcagcaacagcatcaacagcaacagcaacagcagcagcagcagcagcagcagcagcagcagcaacagcagcagcaacaacagcgaccgccacatctggtgcaccacgctgccaaccaccatcccgggcccggggcatggcggagtgcggcggctgcagctcacctccctccctccatgggagcttccaacggcggtttgctctattcgcagccgagcttcacggtgaacggcatgctgggcgcaggagggcagccggctgggctgcaccaccacggcctgagggacgcccacgatgagccacaccatgcagaccaccacccgcatccgcactctcacccacaccagcaaccgcccccgccacctcccccacaaggcccaccgggccacccaggcgcgcaccacgacccgcactcggacgaggacacgccgacctcagacgacctggagcagttcgccaagcaattcaagcagaggcggatcaaactcggatttactcaagcagacgtggggctggcgcttggcaccctgtacggcaacgtgttctcgcagaccaccatctgcaggtttgaggccctgcagctgagcttcaagaacatgtgcaagctgaagcctttgttgaacaagtggttggaagaggcagactcatcctcgggcagccccaccagcatagacaagatcgcagcgcaagggcgcaaacggaaaaagcggacctccatcgaggtgagcgtcaagggggctctggagagccatttcctcaaatgccctaagccctcggcccaggagatcacctccctcgcggacagcttacagctggagaaggaggtggtgagagtttggttttgtaacaggagacagaaagagaaaaggatgacccctcccggagggactctgccgggcgccgaggatgtgtatgggggtagtagggacacgccaccacaccacggggtgcagacgcccgtccagtga

SEQ ID NO: 9 - protein, 236 aa, Homo sapiens
MESSAKMESGGAGQQPQPQPQQPFLPPAACFFATAAAAAAAAAAAAAQSAQQQQQQQQQQQQAPQLRPAADGQPSGGGHKSAPKQVKRQRSSSPELMRCKRRLNFSGFGYSLPQQQPAAVARRNERERNRVKLVNLGFATLREHVPNGAANKKMSKVETLRSAVEYIRALQQLLDEHDAVSAAFQAGVLSPTISPNYSNDLNSMAGSPVSSYSSDEGSYDPLSPEEQELLDFTNWF

SEQ ID NO: 10 - protein, 231 aa, Mus musculus
MESSGKMESGAGQQPQPPQPFLPPAACFFATAAAAAAAAAAAAQSAQQQQPQAPPQQAPQLSPVADSQPSGGGHKSAAKQVKRQRSSSPELMRCKRRLNFSGFGYSLPQQQPAAVARRNERERNRVKLVNLGFATLREHVPNGAANKKMSKVETLRSAVEYIRALQQLLDEHDAVSAAFQAGVLSPTISPNYSNDLNSMAGSPVSSYSSDEGSYDPLSPEEQELLDFTNWF

SEQ ID NO: 11 - DNA, 711 bp, Homo sapiens
  source 1..711: mol_type = genomic DNA
atggaaagctctgccaagatggagagcggcggcgccggccagcagccccagccgcagccccagcagcccttcctgccgcccgcagcctgtttctttgccacggccgcagccgcggcggccgcagccgccgcagcggcagcgcagagcgcgcagcagcagcagcagcagcagcagcagcagcagcaggcgccgcagctgagaccggcggccgacggccagccctcagggggcggtcacaagtcagcgcccaagcaagtcaagcgacagcgctcgtcttcgcccgaactgatgcgctgcaaacgccggctcaacttcagcggctttggctacagcctgccgcagcagcagccggccgccgtggcgcgccgcaacgagcgcgagcgcaaccgcgtcaagttggtcaacctgggctttgccacccttcgggagcacgtccccaacggcgcggccaacaagaagatgagtaaggtggagacactgcgctcggcggtcgagtacatccgcgcgctgcagcagctgctggacgagcatgacgcggtgagcgccgccttccaggcaggcgtcctgtcgcccaccatctcccccaactactccaacgacttgaactccatggccggctcgccggtctcatcctactcgtcggacgagggctcttacgacccgctcagccccgaggagcaggagcttctcgacttcaccaactggttctga

SEQ ID NO: 12 - DNA, 696 bp, Mus musculus
  source 1..696: mol_type = genomic DNA
atggagagctctggcaagatggagagtggagccggccagcagccgcagcccccgcagcccttcctgcctcccgcagcctgcttctttgcgaccgcggcggcggcggcagcggcggcggccgcggcagctcagagcgcgcagcagcaacagccgcaggcgccgccgcagcaggcgccgcagctgagcccggtggccgacagccagccctcagggggcggtcacaagtcagcggccaagcaggtcaagcgccagcgctcgtcctctccggaactgatgcgctgcaaacgccggctcaacttcagcggcttcggctacagcctgccacagcagcagccggccgccgtggcgcgccgcaacgagcgcgagcgcaaccgggtcaagttggtcaacctgggttttgccaccctccgggagcatgtccccaacggcgcggccaacaagaagatgagcaaggtggagacgctgcgctcggcggtcgagtacatccgcgcgctgcagcagctgctggacgagcacgacgcggtgagcgctgcctttcaggcgggcgtcctgtcgcccaccatctcccccaactactccaacgacttgaactctatggcgggttctccggtctcgtcctactcctccgacgagggatcctacgaccctcttagcccagaggaacaagagctgctggactttaccaactggttctga

SEQ ID NO: 13 - protein, 272 aa, Homo sapiens
MFVKSETLELKEEEDVLVLLGSASPALAALTPLSSSADEEEEEEPGASGGARRQRGAEAGQGARGGVAAGAEGCRPARLLGLVHDCKRRPSRARAVSRGAKTAETVQRIKKTRRLKANNRERNRMHNLNAALDALREVLPTFPEDAKLTKIETLRFAHNYIWALTETLRLADHCGGGGGGLPGALFSEAVLLSPGGASAALSSSGDSPSPASTWSCTNSPAPSSSVSSNSTSPYSCTLSPASPAGSDMDYWQPPPPDKHRYAPHLPIARDCI

SEQ ID NO: 14 - protein, 263 aa, Mus musculus
MFVKSETLELKEEEEVLMLLGSASPASATLTPMSSSADEEEDEELRRPGSARGQRGAEAGQGVQGSPASGAGGCRPGRLLGLMHECKRRPSRSRAVSRGAKTAETVQRIKKTRRLKANNRERNRMHNLNAALDALREVLPTFPEDAKLTKIETLRFAHNYIWALTETLRLADHCAGAGGLQGALFTEAVLLSPGAALGASGDSPSPPSSWSCTNSPASSSNSTSPYSCTLSPASPGSDVDYWQPPPPEKHRYAPHLPLARDCI

SEQ ID NO: 15 - DNA, 819 bp, Homo sapiens
  source 1..819: mol_type = genomic DNA
atgttcgtcaaatccgagaccttggagttgaaggaggaagaggacgtgttagtgctgctcggatcggcctcccccgccttggcggccctgaccccgctgtcatccagcgccgacgaagaagaggaggaggagccgggcgcgtcaggcggggcgcgtcggcagcgcggggctgaggccgggcagggggcgcggggcggcgtggctgcgggtgcggagggctgccggcccgcacggctgctgggtctggtacacgattgcaaacggcgcccttcccgggcgcgggccgtctcccgaggcgccaagacggccgagacggtgcagcgcatcaagaagacccgtagactgaaggccaacaaccgcgagcgaaaccgcatgcacaacctcaacgcggcactggacgcgctgcgcgaggtgctccccacgttccccgaggacgccaagctcaccaagatcgagaccctgcgcttcgcccacaactacatctgggcactcaccgagaccctgcgcctggcggatcactgcgggggcggcggcgggggcctgccgggggcgctcttctccgaggcagtgttgctgagcccgggaggagccagcgccgccctgagcagcagcggagacagcccctcgcccgcctccacgtggagttgcaccaacagccccgcgccgtcctcctccgtgtcctccaattccacctccccctacagctgcactttatcgcccgccagcccggccgggtcagacatggactattggcagcccccacctcccgacaagcaccgctatgcacctcacctccccatagccagggattgtatctag

SEQ ID NO: 16 - DNA, 792 bp, Mus musculus
  source 1..792: mol_type = genomic DNA
atgttcgtcaaatctgagactctggagttgaaggaggaagaggaggtactgatgctgctgggctcggcttccccggcctcggcgaccctgaccccgatgtcctccagcgcggacgaggaggaggacgaggagctgcgccggccgggctccgcgcgtgggcagcgtggagcggaagccgggcagggggtgcagggcagtccggcgtcgggtgccgggggttgccggccagggcggctgctgggcctgatgcacgagtgcaagcgtcgcccgtcgcgctcacgggccgtctcccgaggtgccaagacggcggagacggtgcagcgcatcaagaagacccgcaggctcaaggccaacaaccgcgagcgcaaccgcatgcacaacctaaacgccgcgctggacgcgctgcgcgaggtgctgcccaccttccccgaggatgccaagctcacgaagatcgagacgctgcgcttcgcccacaattacatctgggcgctcaccgagactctgcgcctggcggaccactgcgccggcgccggtggcctccagggggcgctcttcacggaggcggtgctcctgagcccgggagctgcgctcggcgccagcggggacagcccttctccaccttcctcctggagctgcaccaacagcccggcgtcatcctccaactccacgtccccatacagctgcactttatcgcccgctagccccgggtcagacgtggactactggcagcccccacctccggagaagcatcgttatgcgcctcacctgcccctcgccagggactgtatctag

SEQ ID NO: 17 - DNA, 2209 bp, Homo sapiens
  source 1..2209: mol_type = other DNA
taatcccacctccctctctgtgctgggactcacagagggagacctcaggaggcagtctgtccatcacatgtccaaatgcagagcataccctgggctgggcgcagtggcgcacaactgtaattccagcactttgggaggctgatgtggaaggatcacttgagcccagaagttctagaccagcctgggcaacatggcaagaccctatctctacaaaaaaagttaaaaaatcagccacgtgtggtgacacacacctgtagtcccagctattcaggaggctgaggtgaggggatcacttaaggctgggaggttgaggctgcagtgagtcgtggttgcgccactgcactccagcctgggcaacagtgagaccctgtctcaaaagacaaaaaaaaaaaaaaaaaaaaaagaacatatcctggtgtggagtaggggacgctgctctgacagaggctcgggggcctgagctggctctgtgagctggggaggaggcagacagccaggccttgtctgcaagcagacctggcagcattgggctggccgccccccagggcctcctcttcatgcccagtgaatgactcaccttggcacagacacaatgttcggggtgggcacagtgcctgcttcccgccgcaccccagcccccctcaaatgccttccgagaagcccattgagcagggggcttgcattgcaccccagcctgacagcctggcatcttgggataaaagcagcacagccccctaggggctgcccttgctgtgtggcgccaccggcggtggagaacaaggctctattcagcctgtgcccaggaaaggggatcaggggatgcccaggcatggacagtgggtggcagggggggagaggagggctgtctgcttcccagaagtccaaggacacaaatgggtgaggggactgggcagggttctgaccctgtgggaccagagtggagggcgtagatggacctgaagtctccagggacaacagggcccaggtctcaggctcctagttgggcccagtggctccagcgtttccaaacccatccatccccagaggttcttcccatctctccaggctgatgtgtgggaactcgaggaaataaatctccagtgggagacggaggggtggccagggaaacggggcgctgcaggaataaagacgagccagcacagccagctcatgtgtaacggctttgtggagctgtcaaggcctggtctctgggagagaggcacagggaggccagacaaggaaggggtgacctggagggacagatccaggggctaaagtcctgataaggcaagagagtgccggccccctcttgccctatcaggacctccactgccacatagaggccatgattgacccttagacaaagggctggtgtccaatcccagcccccagccccagaactccagggaatgaatgggcagagagcaggaatgtgggacatctgtgttcaagggaaggactccaggagtctgctgggaatgaggcctagtaggaaatgaggtggcccttgagggtacagaacaggttcattcttcgccaaattcccagcaccttgcaggcacttacagctgagtgagataatgcctgggttatgaaatcaaaaagttggaaagcaggtcagaggtcatctggtacagcccttccttcccttttttttttttttttttgtgagacaaggtctctctctgttgcccaggctggagtggcgcaaacacagctcactgcagcctcaacctactgggctcaagcaatcctccagcctcagcctcccaaagtgctgggattacaagcatgagccaccccactcagccctttccttcctttttaattgatgcataataattgtaagtattcatcatggtccaaccaaccctttcttgacccaccttcctagagagagggtcctcttgcttcagcggtcagggccccagacccatggtctggctccaggtaccacctgcctcatgcaggagttggcgtgcccaggaagctctgcctctgggcacagtgacctcagtggggtgaggggagctctccccatagctgggctgcggcccaaccccaccccctcaggctatgccagggggtgttgccaggggcacccgggcatcgccagtctagcccactccttcataaagccctcgcatcccaggagcgagcagagccagagcaggttggagaggagacgcatcacctccgctgctcgcgg

SEQ ID NO: 18 - protein, 236 aa, synthetic construct
MESSAKMESGGAGQQPQPQPQQPFLPPAACFFATAAAAAAAAAAAAAQSAQQQQQQQQQQQQAPQLRPAADGQPSGGGHKSAPKQVKRQRSSAPELMRCKRRLNFSGFGYSLPQQQPAAVARRNERERNRVKLVNLGFATLREHVPNGAANKKMSKVETLRSAVEYIRALQQLLDEHDAVSAAFQAGVLAPTIAPNYSNDLNSMAGAPVSSYSSDEGSYDPLAPEEQELLDFTNWF

SEQ ID NO: 19 - DNA, 711 bp, synthetic construct
  source 1..711: mol_type = other DNA
atggaaagctctgccaagatggagagcggcggcgccggccagcagccccagccgcagccccagcagcccttcctgccgcccgcagcctgtttctttgccacggccgcagccgcggcggccgcagccgccgcagcggcagcgcagagcgcgcagcagcagcagcagcagcagcagcagcagcagcaggcgccgcagctgagaccggcggccgacggccagccctcagggggcggtcacaagtcagcgcccaagcaagtcaagcgacagcgctcgtctgcacccgaactgatgcgctgcaaacgccggctcaacttcagcggctttggctacagcctgccgcagcagcagccggccgccgtggcgcgccgcaacgagcgcgagcgcaaccgcgtcaagttggtcaacctgggctttgccacccttcgggagcacgtccccaacggcgcggccaacaagaagatgagtaaggtggagacactgcgctcggcggtcgagtacatccgcgcgctgcagcagctgctggacgagcatgacgcggtgagcgccgccttccaggcaggcgtcctggcacccaccatcgcacccaactactccaacgacttgaactccatggccggcgcaccggtctcatcctactcgtcggacgagggctcttacgacccgctcgcacccgaggagcaggagcttctcgacttcaccaactggttctga